European Patent Application EP 4 331 631 A1, published March 6, 2024. Title: CHIMERIC PEPTIDE-MODIFIED SIS MEMBRANE, PREPARATION METHOD THEREFOR AND APPLICATION THEREOF. Applicant: Beijing Biosis Healing Biological Technology Co., Ltd. The sequence listing filed with the application follows.

SEQUENCE LISTING (32 sequences)

SEQ ID NO: 1 - protein, 29 aa, Artificial Sequence
  sequence of the chimeric peptide
TKKTLRTGGGGSGGGGSKFHEKHHSHRGY

SEQ ID NO: 2 - protein, 31 aa, Artificial Sequence
  sequence of the chimeric peptide
TKKTLRTGGGGSGGGGSKRLFRRLLFSMKKY

SEQ ID NO: 3 - protein, 29 aa, Artificial Sequence
  sequence of the chimeric peptide
KELNLVYGGGGSGGGGSKFHEKHHSHRGY

SEQ ID NO: 4 - protein, 31 aa, Artificial Sequence
  sequence of the chimeric peptide
KELNLVYGGGGSGGGGSKRLFRRLLFSMKKY

SEQ ID NO: 5 - protein, 30 aa, Artificial Sequence
  sequence of the chimeric peptide
TKKTLRTGGGGSGGGGSRKFHEKHHSHRGY

SEQ ID NO: 6 - protein, 30 aa, Artificial Sequence
  sequence of the chimeric peptide
TKKTLRTGGGGSGGGGSFKCKKVVISLRRY

SEQ ID NO: 7 - protein, 30 aa, Artificial Sequence
  sequence of the chimeric peptide
KELNLVYGGGGSGGGGSRKFHEKHHSHRGY

SEQ ID NO: 8 - protein, 30 aa, Artificial Sequence
  sequence of the chimeric peptide
KELNLVYGGGGSGGGGSFKCKKVVISLRRY

SEQ ID NO: 9 - protein, 30 aa, Artificial Sequence
  sequence of the chimeric peptide
TKKTLRTGGGGSGGGGSSHREFPFYGDYGS

SEQ ID NO: 10 - protein, 31 aa, Artificial Sequence
  sequence of the chimeric peptide
TKKTLRTGGGGSGGGGSKRLFRRWQWRMKKY

SEQ ID NO: 11 - protein, 30 aa, Artificial Sequence
  sequence of the chimeric peptide
KELNLVYGGGGSGGGGSSHREFPFYGDYGS

SEQ ID NO: 12 - protein, 31 aa, Artificial Sequence
  sequence of the chimeric peptide
KELNLVYGGGGSGGGGSKRLFRRWQWRMKKY

SEQ ID NO: 13 - protein, 30 aa, Artificial Sequence
  sequence of the chimeric peptide
TKKTLRTEAAAKEAAAKSHREFPFYGDYGS

SEQ ID NO: 14 - protein, 31 aa, Artificial Sequence
  sequence of the chimeric peptide
TKKTLRTEAAAKEAAAKKRLFRRWQWRMKKY

SEQ ID NO: 15 - protein, 30 aa, Artificial Sequence
  sequence of the chimeric peptide
KELNLVYEAAAKEAAAKSHREFPFYGDYGS

SEQ ID NO: 16 - protein, 31 aa, Artificial Sequence
  sequence of the chimeric peptide
KELNLVYEAAAKEAAAKKRLFRRWQWRMKKY

SEQ ID NO: 17 - DNA, 19 bp, Artificial Sequence
  Primer Sequence
tgcggtctcctaaaggtcg

SEQ ID NO: 18 - DNA, 20 bp, Artificial Sequence
  Primer Sequence
actcaaactcgctgaggacg

SEQ ID NO: 19 - DNA, 20 bp, Artificial Sequence
  Primer Sequence
ccgaactggtccgcaccgac

SEQ ID NO: 20 - DNA, 20 bp, Artificial Sequence
  Primer Sequence
cttgaaggccacgggcaggg

SEQ ID NO: 21 - DNA, 18 bp, Artificial Sequence
  Primer Sequence
aggcaggattgaccacgg

SEQ ID NO: 22 - DNA, 18 bp, Artificial Sequence
  Primer Sequence
tgtagttctgctcatgga

SEQ ID NO: 23 - DNA, 17 bp, Artificial Sequence
  Primer Sequence
aatgaagggccctgagc

SEQ ID NO: 24 - DNA, 19 bp, Artificial Sequence
  Primer Sequence
gccagttctgcaaggaagc

SEQ ID NO: 25 - DNA, 21 bp, Artificial Sequence
  Primer Sequence
gacggccgcatcttcttgtgc

SEQ ID NO: 26 - DNA, 21 bp, Artificial Sequence
  Primer Sequence
tgcaaatggcagccctggtga

SEQ ID NO: 27 - DNA, 22 bp, Artificial Sequence
  Primer Sequence
cctacttctgcacgatgtgatg

SEQ ID NO: 28 - DNA, 23 bp, Artificial Sequence
  Primer Sequence
cctttgctacggttggttacatt

SEQ ID NO: 29 - DNA, 21 bp, Artificial Sequence
  Primer Sequence
ctaccacaacgagatgtgcaa

SEQ ID NO: 30 - DNA, 21 bp, Artificial Sequence
  Primer Sequence
ccgaagtacacagtgttctgg

SEQ ID NO: 31 - DNA, 21 bp, Artificial Sequence
  Primer Sequence
ggagcgagatccctccaaaat

SEQ ID NO: 32 - DNA, 23 bp, Artificial Sequence
  Primer Sequence
ggctgttgtcatacttctcatgg